European Patent Specification EP 2 506 881 B1, published March 6, 2024. Title: COMBINING RADIOIMMUNOTHERAPY AND ANTIBODY-DRUG CONJUGATES FOR IMPROVED CANCER THERAPY. Applicant: IMMUNOMEDICS, INC. The sequence listing filed with the application follows.

SEQUENCE LISTING (60 sequences)

SEQ ID NO: 1 - protein, 12 aa, Artificial Sequence
  Description of Artificial Sequence: Synthetic peptide
SASSSVSSSYLY

SEQ ID NO: 2 - protein, 7 aa, Artificial Sequence
  Description of Artificial Sequence: Synthetic peptide
STSNLAS

SEQ ID NO: 3 - protein, 9 aa, Artificial Sequence
  Description of Artificial Sequence: Synthetic peptide
HQWNRYPYT

SEQ ID NO: 4 - protein, 5 aa, Artificial Sequence
  Description of Artificial Sequence: Synthetic peptide
SYVLH

SEQ ID NO: 5 - protein, 17 aa, Artificial Sequence
  Description of Artificial Sequence: Synthetic peptide
YINPYNDGTQYNEKFKG

SEQ ID NO: 6 - protein, 10 aa, Artificial Sequence
  Description of Artificial Sequence: Synthetic peptide
GFGGSYGFAY

SEQ ID NO: 7 - protein, 11 aa, Artificial Sequence
  Description of Artificial Sequence: Synthetic peptide
KASQDVSIAVA

SEQ ID NO: 8 - protein, 7 aa, Artificial Sequence
  Description of Artificial Sequence: Synthetic peptide
SASYRYT

SEQ ID NO: 9 - protein, 9 aa, Artificial Sequence
  Description of Artificial Sequence: Synthetic peptide
QQHYITPLT

SEQ ID NO: 10 - protein, 5 aa, Artificial Sequence
  Description of Artificial Sequence: Synthetic peptide
NYGMN

SEQ ID NO: 11 - protein, 17 aa, Artificial Sequence
  Description of Artificial Sequence: Synthetic peptide
WINTYTGEPTYTDDFKG

SEQ ID NO: 12 - protein, 12 aa, Artificial Sequence
  Description of Artificial Sequence: Synthetic peptide
GGFGSSYWYFDV

SEQ ID NO: 13 - protein, 44 aa, Artificial Sequence
  Description of Artificial Sequence: Synthetic polypeptide
SHIQIPPGLTELLQGYTVEVLRQQPPDLVEFAVEYFTRLREARA

SEQ ID NO: 14 - protein, 45 aa, Artificial Sequence
  Description of Artificial Sequence: Synthetic polypeptide
CGHIQIPPGLTELLQGYTVEVLRQQPPDLVEFAVEYFTRLREARA

SEQ ID NO: 15 - protein, 17 aa, Artificial Sequence
  Description of Artificial Sequence: Synthetic peptide
QIEYLAKQIVDNAIQQA

SEQ ID NO: 16 - protein, 21 aa, Artificial Sequence
  Description of Artificial Sequence: Synthetic peptide
CGQIEYLAKQIVDNAIQQAGC

SEQ ID NO: 17 - protein, 50 aa, Artificial Sequence
  Description of Artificial Sequence: Synthetic polypeptide
SLRECELYVQKHNIQALLKDSIVQLCTARPERPMAFLREYFERLEKEEAK

SEQ ID NO: 18 - protein, 55 aa, Artificial Sequence
  Description of Artificial Sequence: Synthetic polypeptide
MSCGGSLRECELYVQKHNIQALLKDSIVQLCTARPERPMAFLREYFERLEKEEAK

SEQ ID NO: 19 - protein, 23 aa, Artificial Sequence
  Description of Artificial Sequence: Synthetic peptide
CGFEELAWKIAKMIWSDVFQQGC

SEQ ID NO: 20 - protein, 55 aa, Artificial Sequence
  Description of Artificial Sequence: Synthetic polypeptide
GSGGGGSGGGGSHIQIPPGLTELLQGYTVEVLRQQPPDLVEFAVEYFTRLREARA

SEQ ID NO: 21 - protein, 29 aa, Artificial Sequence
  Description of Artificial Sequence: Synthetic peptide
GSGGGGSGGGGSQIEYLAKQIVDNAIQQA

SEQ ID NO: 22 - protein, 51 aa, Homo sapiens
SLRECELYVQKHNIQALLKDVSIVQLCTARPERPMAFLREYFEKLEKEEAK

SEQ ID NO: 23 - protein, 54 aa, Homo sapiens
SLKGCELYVQLHGIQQVLKDCIVHLCISKPERPMKFLREHFEKLEKEENRQILA

SEQ ID NO: 24 - protein, 44 aa, Homo sapiens
SHIQIPPGLTELLQGYTVEVGQQPPDLVDFAVEYFTRLREARRQ

SEQ ID NO: 25 - protein, 44 aa, Homo sapiens
SIEIPAGLTELLQGFTVEVLRHQPADLLEFALQHFTRLQQENER

SEQ ID NO: 26 - protein, 17 aa, Artificial Sequence
  Description of Artificial Sequence: Synthetic peptide
QIEYVAKQIVDYAIHQA

SEQ ID NO: 27 - protein, 17 aa, Artificial Sequence
  Description of Artificial Sequence: Synthetic peptide
QIEYKAKQIVDHAIHQA

SEQ ID NO: 28 - protein, 17 aa, Artificial Sequence
  Description of Artificial Sequence: Synthetic peptide
QIEYHAKQIVDHAIHQA

SEQ ID NO: 29 - protein, 17 aa, Artificial Sequence
  Description of Artificial Sequence: Synthetic peptide
QIEYVAKQIVDHAIHQA

SEQ ID NO: 30 - protein, 18 aa, Artificial Sequence
  Description of Artificial Sequence: Synthetic peptide
PLEYQAGLLVQNAIQQAI

SEQ ID NO: 31 - protein, 18 aa, Artificial Sequence
  Description of Artificial Sequence: Synthetic peptide
LLIETASSLVKNAIQLSI

SEQ ID NO: 32 - protein, 18 aa, Artificial Sequence
  Description of Artificial Sequence: Synthetic peptide
LIEEAASRIVDAVIEQVK

SEQ ID NO: 33 - protein, 18 aa, Artificial Sequence
  Description of Artificial Sequence: Synthetic peptide
ALYQFADRFSELVISEAL

SEQ ID NO: 34 - protein, 17 aa, Artificial Sequence
  Description of Artificial Sequence: Synthetic peptide
LEQVANQLADQIIKEAT

SEQ ID NO: 35 - protein, 17 aa, Artificial Sequence
  Description of Artificial Sequence: Synthetic peptide
FEELAWKIAKMIWSDVF

SEQ ID NO: 36 - protein, 18 aa, Artificial Sequence
  Description of Artificial Sequence: Synthetic peptide
ELVRLSKRLVENAVLKAV

SEQ ID NO: 37 - protein, 18 aa, Artificial Sequence
  Description of Artificial Sequence: Synthetic peptide
TAEEVSARIVQVVTAEAV

SEQ ID NO: 38 - protein, 18 aa, Artificial Sequence
  Description of Artificial Sequence: Synthetic peptide
QIKQAAFQLISQVILEAT

SEQ ID NO: 39 - protein, 16 aa, Artificial Sequence
  Description of Artificial Sequence: Synthetic peptide
LAWKIAKMIVSDVMQQ

SEQ ID NO: 40 - protein, 24 aa, Artificial Sequence
  Description of Artificial Sequence: Synthetic peptide
DLIEEAASRIVDAVIEQVKAAGAY

SEQ ID NO: 41 - protein, 18 aa, Artificial Sequence
  Description of Artificial Sequence: Synthetic peptide
LEQYANQLADQIIKEATE

SEQ ID NO: 42 - protein, 20 aa, Artificial Sequence
  Description of Artificial Sequence: Synthetic peptide
FEELAWKIAKMIWSDVFQQC

SEQ ID NO: 43 - protein, 17 aa, Artificial Sequence
  Description of Artificial Sequence: Synthetic peptide
QIEYLAKQIPDNAIQQA

SEQ ID NO: 44 - protein, 25 aa, Artificial Sequence
  Description of Artificial Sequence: Synthetic peptide
KGADLIEEAASRIVDAVIEQVKAAG

SEQ ID NO: 45 - protein, 25 aa, Artificial Sequence
  Description of Artificial Sequence: Synthetic peptide
KGADLIEEAASRIPDAPIEQVKAAG

SEQ ID NO: 46 - protein, 25 aa, Artificial Sequence
  Description of Artificial Sequence: Synthetic peptide
PEDAELVRLSKRLVENAVLKAVQQY

SEQ ID NO: 47 - protein, 25 aa, Artificial Sequence
  Description of Artificial Sequence: Synthetic peptide
PEDAELVRTSKRLVENAVLKAVQQY

SEQ ID NO: 48 - protein, 25 aa, Artificial Sequence
  Description of Artificial Sequence: Synthetic peptide
PEDAELVRLSKRDVENAVLKAVQQY

SEQ ID NO: 49 - protein, 25 aa, Artificial Sequence
  Description of Artificial Sequence: Synthetic peptide
PEDAELVRLSKRLPENAVLKAVQQY

SEQ ID NO: 50 - protein, 25 aa, Artificial Sequence
  Description of Artificial Sequence: Synthetic peptide
PEDAELVRLSKRLPENAPLKAVQQY

SEQ ID NO: 51 - protein, 25 aa, Artificial Sequence
  Description of Artificial Sequence: Synthetic peptide
PEDAELVRLSKRLVENAVEKAVQQY

SEQ ID NO: 52 - protein, 25 aa, Artificial Sequence
  Description of Artificial Sequence: Synthetic peptide
EEGLDRNEEIKRAAFQIISQVISEA

SEQ ID NO: 53 - protein, 25 aa, Artificial Sequence
  Description of Artificial Sequence: Synthetic peptide
LVDDPLEYQAGLLVQNAIQQAIAEQ

SEQ ID NO: 54 - protein, 25 aa, Artificial Sequence
  Description of Artificial Sequence: Synthetic peptide
QYETLLIETASSLVKNAIQLSIEQL

SEQ ID NO: 55 - protein, 25 aa, Artificial Sequence
  Description of Artificial Sequence: Synthetic peptide
LEKQYQEQLEEEVAKVIVSMSIAFA

SEQ ID NO: 56 - protein, 25 aa, Artificial Sequence
  Description of Artificial Sequence: Synthetic peptide
NTDEAQEELAWKIAKMIVSDIMQQA

SEQ ID NO: 57 - protein, 25 aa, Artificial Sequence
  Description of Artificial Sequence: Synthetic peptide
VNLDKKAVLAEKIVAEAIEKAEREL

SEQ ID NO: 58 - protein, 25 aa, Artificial Sequence
  Description of Artificial Sequence: Synthetic peptide
NGILELETKSSKLVQNIIQTAVDQF

SEQ ID NO: 59 - protein, 25 aa, Artificial Sequence
  Description of Artificial Sequence: Synthetic peptide
TQDKNYEDELTQVALALVEDVINYA

SEQ ID NO: 60 - protein, 25 aa, Artificial Sequence
  Description of Artificial Sequence: Synthetic peptide
ETSAKDNINIEEAARFLVEKILVNH